European Patent Specification EP 4 150 119 B1, published December 4, 2024. Title: EPIGENETIC MODIFICATION OF SELECT GENES AS MARKERS OF HYPERSOMNOLENCE. Applicant: Wisconsin Alumni Research Foundation. The sequence listing filed with the application follows.

SEQUENCE LISTING (37 sequences)

SEQ ID NO: 1 - DNA, 385 bp, Homo sapiens
cgccgccatagctgcatggccccgggacctccctgtcgtacctgagaggagggcctggcccgtgaactgcccgtacacggaggcagcatggggaaaggcattgaagggcgggaccccggagccgacttgctgcagatccaaaaaggcggagctagataaagaggaaggggtggagctagaactggacacctcgggggtttcctgctttatggcgaagggtgagtgaggatctgccggagggagggagacaacaaggagagaggggtgtgagatggcggggagggaacacgcacaagccaagccgtgggatgtggagggtgcgggcggggcgcggggcaggctcagctgccctcagagtctgggctggggagagccggggcccacg

SEQ ID NO: 2 - DNA, 2528 bp, Homo sapiens
cgccgccatagctgcatggccccgggacctccctgtcgtacctgagaggagggcctggcccgtgaactgcccgtacacggaggcagcatggggaaaggcattgaagggcgggaccccggagccgacttgctgcagatccaaaaaggcggagctagataaagaggaaggggtggagctagaactggacacctcgggggtttcctgctttatggcgaagggtgagtgaggatctgccggagggagggagacaacaaggagagaggggtgtgagatggcggggagggaacacgcacaagccaagccgtgggatgtggagggtgcgggcggggcgcggggcaggctcagctgccctcagagtctgggctggggagagccggggcccacgaggcgtggcaaggcggggagagagaagctagacctccctgctgcgcttctgcagcgaaaatggagagacccggaaggcgtgtgtgcgcccgcctctcccacaggagggagcgcggagacccgggagcggcctaggaccggaggcgcgacccctcggcccaccttgaggcccggcctaggaccggaggcgcgacccctgggcccaccttgaggcccggcctaggactggaggcgcgacccctcggcccaccttgcgggagccgcctaggaccggaggcgcgacccctcggcccagcttgaggcccggcctaggaccggaggcgcgacccctcggcccaccttgcgggagccgcctaggaccggaggcgcgacccctcggcccaccttgaggcccggcctaggaccggaggcgcgacccctgggcccaccttgaggcccggcctaggactggaggcgcgacccctcggcccaccttacgggagccgcctagggccggaggcgcgacccctcggcccagcttgaggcccggcctaggaccggaggcgcgacccctcggcccaccttgaggcccggcctaggactggaggcgcgacccctcggcccaccttgaggcccggcctaggaccggaggcgcgacccctgggcccaccttgaggcccggcctaggactggaggcgcgacccctcggcccaccttgaggcccggcctaggaccggaggcgcgacccctgggcccacctggcggcccggccggcacagcccgcctctcctctccaggccagggccccacaccttccgcctgacagccagccaagctcttcagtcccccgccctccacctgccagggaggctccgggcgttgtacctgccaccacggggtaggtctggtgagtcgagaggttgcgccccagtggcgtgttggaaggggtcagggtggccttcccgtcgtccagggtgctgttgagcaagggcagcgggtagaggccctggggagcaaagagaagtcagcgcacagagacgatccaacaagccgaccttcctgcagaccctgagcctgtgtcttaggacttggcagccctcatctccccaggagaggtcctcatcgcccccttcttcctttacgttctcaactccactcggcacgtttcgttcatgctcattgtcctcccgcatccctggaattcaaggccagctggtagcatgggtgcccagacgtgggatagagagtctcagccagaggaccacaccctggttggatggctggtcggcttcctggtttcaccacactgttgggacccacagaatgcaggacggtgccaaggactggagcagtctccaaccggactgttcagggtccttgcatctgttaatttattcttccccagataggaaacccaggcacaaaggtttaagaaacttgtcccacttccagatgggccaaagataggattcagattcgagggatcagaatgtgtctgctctcaaccactgccctaaactgggtgacataaggaccacttcttacatttgcaaagagcttatatcagagctttgcctctgttgtcctagtagagtcccccagcagcccagtgacatgggtgagtaatattatgtctgtgttttatatgtggagcctggaactcaggtaaatggcccaattttgtatagtgaaacagactaaacccgggatttttcggctgtggacccaggtgctttacccaccacgtggatttcttcttttctctctccacatccaaacaaatagaagtgtgcaagttcggcttgaaaatggtattgagagttgtttttgttggaaacactctttgtcaagtacctgggggtcttcatcagtaagacctcattttagatgcctcctggcctccccttcccaggagcacagctatgaccttaggtactccttccgaaaagaacttgtttaactaaaggtaagtgtacctcatcctcaccatggcctccttccactggggaagcagatagcgcagaaaaaagaacacacccattccccacataccttcacactcgtcacatacctgctacgtgagatgtgcaaagctgaattcagggaatgctcagtagttacataacagtgccactaaaggcaattgttttcagtgatttccatcg

SEQ ID NO: 3 - DNA, 4435 bp, Homo sapiens
cgatcggctttttctttccctttttgtgggttttattatttttgttacaggtggggctgccagggatgggttatgcctgcagggggagaaatgatcagaagagccacaattctaccctcaacccagggaatgtgagcttttactgcctccattttcttaaccagaaatctggtttagttttgctttcagggctcttgtcattggaaaaagattagtgctcagaacctgcagcccagaaatggcccagtcccatccctccaggcaggctctgctcctcaagctgcgtggggaaatgccatcatgggcttgtgcccagcatccaccctgccaatgatgacaacagtgataatcgaggcattcataccaaccaccatttagggagcctttatagagacttccccccaacagtggcctctttggcagctctgggagacagccttggaaagggcgaactaagggccgagagaagcagcaacttgcgaaggtcactactggccagactgggcccagtctcctgcctcttcccacagtggctgcacaccctactctctaccccattgcagtaggaagagaactccagaataaggggaggctctgaacagtggagtcaggatccgtgttttgactagtttcaaggtctagtaaagcacagtatccaaggaggctcagtccagcatgggcatgggctagggctggagaagtagaaaagaaatttgggcaagtagtgaataagactgccaaatctattgttaggagagccaggagaggtgtcctagtggtgccttagtctatgggagagacccagacaccattctgctgggttcccaagctggcaccttaaatttagtagctgatgaatccaaggagcccccaagcatcatctggcatgtttttttgtatgtttgtttgtttgttttttgagacagagtctctctctgttacccaggctggagtgtagtgacgtgatcttggctcaccacaatgtccgcctcccaggttcaagtgattctcttgcctcagcctcctgagtagctgggactacaggcacgtgccaccacacctggctaagttttgtatttttagtagagatgggtttcaccatgttggccaggatggtctcgatctcctgaccttgtgatctaccagccttggcctcccaaagtgctgcgattataggtgtgagccaccacacccggcccatctggcatgttttataccaactggagtcaggcctagagcagggaggtggctagacagtgactgtaacctccatttcctgtcctggccaaaccaatactcagatgggacagtgagaggagacatcacactctggttacacaccattaacccctgtctgactacacacacacacacacacagccgtccagattcacaaatacgttcttatcacccccttcatccctcagtgcctgggtggaggcccttaagcaggaatgccccctcagaggagagggtgggagtggaatgatgggatttcagaatcccctcacctcaccctctcacctccagatcctagtccagatgtaatcctgtcctcaccactttgcgtgcacgtgcacgcacacacacatgcacacacacagtctcaacattcacatacagacacccactcttgacacccacacatgaactaaaagacaaacgttggtccataaaggaacacacatgctatctacatacccccaaccctgcccagtgatgctttccccagcactactgcacagatcccagacaatacagacacacaggcactccttgcacactgagtcctaggccacttggttgagctgcccccaccccaccccagctgcacactcttctacatccatcccataaaggaagagtccgtctctttaaccatgcttctcatggttttcagagtacccttgccccaaatgctgccaacctccccctagactcaagatcttctctttccagatcgctggaggctcaatgccagtgcacaggaggagatcgccttccaccatattccctgactcccagaggctctttctagggcaggggtctggccaggaagactgaagccatgacgtcttcctgtgcaaggataggaaagatgtctgtgggttggagggtagttatagggaagcagctttctccactttttgagaaagcacttgggaacaagcatccctctcaggaagtgattctccaccattctcctctgatcctataggcctggtggtccaagcctcaggccagttgatgcctcccactgggatcagcagacaaggccatgaccctgcagtgacctcgaccccataatcaggtcaggtccgggcttcatggctagaagcgaggcccaggcgagtggccaagacgcggcaggacaggaggatgcgcctggctgctctcggctgctggacgcggcctgcagtagggagagcgcagcccggggtaatcccactcagggctccgggtgcccagttctcccacttcccatcctggcggcctaaaggcaaggcctagaccctggagaggccaaagtcgggccaaaacaacagcgaagctgggactggaacaggcgctgggggcctgcgcatgaccccaggctcagaatgcgacactccagtgacgccggggaatgagttgagatggagccggagacagaggttggggttcaggacgaggcgcttgggtatgggatcggatctgagacggttgcggcgctggtgctttgggctggaccagactcgaacccagagcggagcgagggtcagagccagggcaagagtccgaagcccagctcagcgtccagcccgcgagagaccccaccatgaatgacgtccgagtagggttggaactcgaagcccgaacgcactggaaatgcagccggacgacggctgggatccgagtgggtccgggccagaaatggggacctcagagctccaccgaggcgctcgaggtcagaactgaagcctgagacttaggcaggacccgagacagagccagagacgataccgaaacccaatggaccgcgaggaccgaaggcagatccggggcgcaaacctgtgcaggcactggcgcgctgcctggagctctgggttcgcgccgctgagcgccggcaggttggaccagcgctgcgcgccggaagtgcactcgggacgccggggttctggaggagagaccacacgccgcaaaagtggcctccgaatgcgcccggggcctgccctcggcgacactgctggctcggcggccgcagcctacctgaagtagtccatcttgcagaagatctccttgttcttgatgtagcagctgttctgctgcctcagcgacgtgcgacacacggagcactcgaggcaccgcacgtgccagatgaggttgttgacctggggacggggcggggacggaggtcggctcagcgcgggcctctttcactccgggccccagccttcccggtctcatttacagtcagaggcgctgaagctcagaaggtgcatgcgattcccctatttttctcccgtaatactgagactcagggaaatggaaataaactcttcttatttttcagacggaacccgggggctcaggcagaccctaagtcttgcccaaagcttcgcagtcgggcagcagtggagccaggatttggaagtaagaggacctgcggtgcttccctgcagtctcctgcgctgcgtcccacgccccgacaacacgcacgcaacacctacccctgtctcaccttgagcagatatcggtccaggatctcgaggccgcagctggagcagatgttcttgcctgcagacggcacggaggaggcggcagagggcggtgagcagacagatggcgtgctgggcgtacatggggaggcctgaccctcgtccttgtccagagctcctgccagggcctcggcgtcagactgagcctgcggcgggggagagaaggagaggagcgctgatccgggcacccagagttggggctgccttggagacaaatctggggcccccgagcaccaattgacaacgaaatctccccaggacaatgcgccgtagactgaaggacagggatggaagggcctattggagaggaagggacggccccaacttttaacacgcgcattctgggtgctgggagcggttaaagccaacattccctgccggaaaaccgaggctcagagaggggcggcgcccgccgggagtcccccagagcgtgagcagcagttcgtggccggaaaacctggccaggtccccagggccgggccgctggaggactgggcaccgcaggcagggccaaacggactcaccatggcgggcggcgcggtcccttcaagacagcgggtggtcgctttgcagccggaccctggctgggccatcacctgggggagggggggagggaacgcaggcggcggcggctgctgaactggctccgcacagcctgagcccagcgcctccccgcg

SEQ ID NO: 4 - DNA, 500 bp, Homo sapiens
cggtgcttccctgcagtctcctgcgctgcgtcccacgccccgacaacacgcacgcaacacctacccctgtctcaccttgagcagatatcggtccaggatctcgaggccgcagctggagcagatgttcttgcctgcagacggcacggaggaggcggcagagggcggtgagcagacagatggcgtgctgggcgtacatggggaggcctgaccctcgtccttgtccagagctcctgccagggcctcggcgtcagactgagcctgcggcgggggagagaaggagaggagcgctgatccgggcacccagagttggggctgccttggagacaaatctggggcccccgagcaccaattgacaacgaaatctccccaggacaatgcgccgtagactgaaggacagggatggaagggcctattggagaggaagggacggccccaacttttaacacgcgcattctgggtgctgggagcggttaaagccaacattccctgccggaaaaccg

SEQ ID NO: 5 - DNA, 304 bp, Homo sapiens
cgtttgacagctgctctggagccgaggatcacaataagagaaggcgcgtgaggctccggcagcaaacaccagccaggcaggcagcggtaatcacagtgagcaaagttgaagactataaaagagccaggctaacgtgctgccgagcaggtgtcctggattttattgtagttgcaaatatgcttctggtgataagtatcgaaattattttttaagtgcgctggggaggagggaggtgcgggaattgagcctcctccgtttccagggagcctctgaaagtggggtggggggagatgaggcatgcacg

SEQ ID NO: 6 - DNA, 885 bp, Homo sapiens
aggccaagttgctacgttacagcacccggctcccggccttagggttcctgcttttccatggggtcttggggtggtgcatccccggcacccctacagcatccgccccttccgagcatgtcttccccgtcacagagaacttcatgttggcgcctccaaaagttgccggaggaattagggaacagggtgggggtggatgagactgaggccagagagggggctggcggtctgccctgaggacccccgtcccacccgccgccatagctgcatggccccgggacctccctgtcgtacctgagaggagggcctggcccgtgaactgcccgtacacggaggcagcatggggaaaggcattgaagggcgggaccccggagccgacttgctgcagatccaaaaaggcggagctagataaagaggaaggggtggagctagaactggacacctcgggggtttcctgctttatggcgaagggtgagtgaggatctgccggagggagggagacaacaaggagagaggggtgtgagatggcggggagggaacacgcacaagccaagccgtgggatgtggagggtgcgggcggggcgcggggcaggctcagctgccctcagagtctgggctggggagagccggggcccacgaggcgtggcaaggcggggagagagaagctagacctccctgctgcgcttctgcagcgaaaatggagagacccggaaggcgtgtgtgcgcccgcctctcccacaggagggagcgcggagacccgggagcggcctaggaccggaggcgcgacccctcggcccaccttgaggcccggcctaggaccggaggcgcgacccctgggcccaccttgaggcccggcctaggactggaggcgcgacccctcggcccacc

SEQ ID NO: 7 - DNA, 885 bp, Artificial Sequence
  Bisulfite modified sequence
aggttaagttgttacgttatagtattcggttttcggttttagggtttttgtttttttatggggttttggggtggtgtattttcggtatttttatagtattcgtttttttcgagtatgtttttttcgttatagagaattttatgttggcgtttttaaaagttgtcggaggaattagggaatagggtgggggtggatgagattgaggttagagagggggttggcggtttgttttgaggattttcgttttattcgtcgttatagttgtatggtttcgggatttttttgtcgtatttgagaggagggtttggttcgtgaattgttcgtatacggaggtagtatggggaaaggtattgaagggcgggatttcggagtcgatttgttgtagatttaaaaaggcggagttagataaagaggaaggggtggagttagaattggatatttcgggggttttttgttttatggcgaagggtgagtgaggatttgtcggagggagggagataataaggagagaggggtgtgagatggcggggagggaatacgtataagttaagtcgtgggatgtggagggtgcgggcggggcgcggggtaggtttagttgtttttagagtttgggttggggagagtcggggtttacgaggcgtggtaaggcggggagagagaagttagatttttttgttgcgtttttgtagcgaaaatggagagattcggaaggcgtgtgtgcgttcgttttttttataggagggagcgcggagattcgggagcggtttaggatcggaggcgcgatttttcggtttattttgaggttcggtttaggatcggaggcgcgatttttgggtttattttgaggttcggtttaggattggaggcgcgatttttcggtttatt

SEQ ID NO: 8 - DNA, 20 bp, Artificial Sequence
  Primer
gaggttagagagggggttgg

SEQ ID NO: 9 - DNA, 20 bp, Artificial Sequence
  Primer
cgctacaaaaacgcaacaaa

SEQ ID NO: 10 - DNA, 1922 bp, Homo sapiens
ccttacgggagccgcctagggccggaggcgcgacccctcggcccagcttgaggcccggcctaggaccggaggcgcgacccctcggcccaccttgaggcccggcctaggactggaggcgcgacccctcggcccaccttgaggcccggcctaggaccggaggcgcgacccctgggcccaccttgaggcccggcctaggactggaggcgcgacccctcggcccaccttgaggcccggcctaggaccggaggcgcgacccctgggcccacctggcggcccggccggcacagcccgcctctcctctccaggccagggccccacaccttccgcctgacagccagccaagctcttcagtcccccgccctccacctgccagggaggctccgggcgttgtacctgccaccacggggtaggtctggtgagtcgagaggttgcgccccagtggcgtgttggaaggggtcagggtggccttcccgtcgtccagggtgctgttgagcaagggcagcgggtagaggccctggggagcaaagagaagtcagcgcacagagacgatccaacaagccgaccttcctgcagaccctgagcctgtgtcttaggacttggcagccctcatctccccaggagaggtcctcatcgcccccttcttcctttacgttctcaactccactcggcacgtttcgttcatgctcattgtcctcccgcatccctggaattcaaggccagctggtagcatgggtgcccagacgtgggatagagagtctcagccagaggaccacaccctggttggatggctggtcggcttcctggtttcaccacactgttgggacccacagaatgcaggacggtgccaaggactggagcagtctccaaccggactgttcagggtccttgcatctgttaatttattcttccccagataggaaacccaggcacaaaggtttaagaaacttgtcccacttccagatgggccaaagataggattcagattcgagggatcagaatgtgtctgctctcaaccactgccctaaactgggtgacataaggaccacttcttacatttgcaaagagcttatatcagagctttgcctctgttgtcctagtagagtcccccagcagcccagtgacatgggtgagtaatattatgtctgtgttttatatgtggagcctggaactcaggtaaatggcccaattttgtatagtgaaacagactaaacccgggatttttcggctgtggacccaggtgctttacccaccacgtggatttcttcttttctctctccacatccaaacaaatagaagtgtgcaagttcggcttgaaaatggtattgagagttgtttttgttggaaacactctttgtcaagtacctgggggtcttcatcagtaagacctcattttagatgcctcctggcctccccttcccaggagcacagctatgaccttaggtactccttccgaaaagaacttgtttaactaaaggtaagtgtacctcatcctcaccatggcctccttccactggggaagcagatagcgcagaaaaaagaacacacccattccccacataccttcacactcgtcacatacctgctacgtgagatgtgcaaagctgaattcagggaatgctcagtagttacataacagtgccactaaaggcaattgttttcagtgatttccatcgagctgggttctgcaaagatccacagcactttccggttgcatgctgggcacttttggaagctgcagtcaattctggaggccaccagggcaccattagcacatagcagcaattattgactaaatggtgctctggttccatgccttccaagggggcccacttagaggcagggtggagttgcttagggcctttttttttttttttttttgtagacggagttttgctcttgttgcccaagctggagtgcaatgg

SEQ ID NO: 11 - DNA, 1922 bp, Artificial Sequence
  Bisulfite modified sequence
ttttacgggagtcgtttagggtcggaggcgcgatttttcggtttagtttgaggttcggtttaggatcggaggcgcgatttttcggtttattttgaggttcggtttaggattggaggcgcgatttttcggtttattttgaggttcggtttaggatcggaggcgcgatttttgggtttattttgaggttcggtttaggattggaggcgcgatttttcggtttattttgaggttcggtttaggatcggaggcgcgatttttgggtttatttggcggttcggtcggtatagttcgttttttttttttaggttagggttttatatttttcgtttgatagttagttaagttttttagtttttcgttttttatttgttagggaggtttcgggcgttgtatttgttattacggggtaggtttggtgagtcgagaggttgcgttttagtggcgtgttggaaggggttagggtggttttttcgtcgtttagggtgttgttgagtaagggtagcgggtagaggttttggggagtaaagagaagttagcgtatagagacgatttaataagtcgatttttttgtagattttgagtttgtgttttaggatttggtagtttttatttttttaggagaggtttttatcgtttttttttttttttacgtttttaattttattcggtacgtttcgtttatgtttattgttttttcgtatttttggaatttaaggttagttggtagtatgggtgtttagacgtgggatagagagttttagttagaggattatattttggttggatggttggtcggttttttggttttattatattgttgggatttatagaatgtaggacggtgttaaggattggagtagtttttaatcggattgtttagggtttttgtatttgttaatttatttttttttagataggaaatttaggtataaaggtttaagaaatttgttttatttttagatgggttaaagataggatttagattcgagggattagaatgtgtttgtttttaattattgttttaaattgggtgatataaggattattttttatatttgtaaagagtttatattagagttttgtttttgttgttttagtagagttttttagtagtttagtgatatgggtgagtaatattatgtttgtgttttatatgtggagtttggaatttaggtaaatggtttaattttgtatagtgaaatagattaaattcgggatttttcggttgtggatttaggtgttttatttattacgtggatttttttttttttttttttatatttaaataaatagaagtgtgtaagttcggtttgaaaatggtattgagagttgtttttgttggaaatattttttgttaagtatttgggggtttttattagtaagattttattttagatgttttttggttttttttttttaggagtatagttatgattttaggtatttttttcgaaaagaatttgtttaattaaaggtaagtgtattttatttttattatggtttttttttattggggaagtagatagcgtagaaaaaagaatatatttattttttatatatttttatattcgttatatatttgttacgtgagatgtgtaaagttgaatttagggaatgtttagtagttatataatagtgttattaaaggtaattgtttttagtgatttttatcgagttgggttttgtaaagatttatagtatttttcggttgtatgttgggtatttttggaagttgtagttaattttggaggttattagggtattattagtatatagtagtaattattgattaaatggtgttttggttttatgttttttaagggggtttatttagaggtagggtggagttgtttagggtttttttttttttttttttttgtagacggagttttgtttttgttgtttaagttggagtgtaatgg

SEQ ID NO: 12 - DNA, 18 bp, Artificial Sequence
  Primer
tacgggagtcgtttaggg

SEQ ID NO: 13 - DNA, 18 bp, Artificial Sequence
  Primer
ctcaacaacaccctaaac

SEQ ID NO: 14 - DNA, 20 bp, Artificial Sequence
  Primer
attttggttggatggttggt

SEQ ID NO: 15 - DNA, 20 bp, Artificial Sequence
  Primer
acaaccgaaaaatcccgaat

SEQ ID NO: 16 - DNA, 23 bp, Artificial Sequence
  Primer
tggggaagtagatagcgtagaaa

SEQ ID NO: 17 - DNA, 22 bp, Artificial Sequence
  Primer
ccctaaacaactccaccctacc

SEQ ID NO: 18 - DNA, 1000 bp, Homo sapiens
cggctcagcgcgggcctctttcactccgggccccagccttcccggtctcatttacagtcagaggcgctgaagctcagaaggtgcatgcgattcccctatttttctcccgtaatactgagactcagggaaatggaaataaactcttcttatttttcagacggaacccgggggctcaggcagaccctaagtcttgcccaaagcttcgcagtcgggcagcagtggagccaggatttggaagtaagaggacctgcggtgcttccctgcagtctcctgcgctgcgtcccacgccccgacaacacgcacgcaacacctacccctgtctcaccttgagcagatatcggtccaggatctcgaggccgcagctggagcagatgttcttgcctgcagacggcacggaggaggcggcagagggcggtgagcagacagatggcgtgctgggcgtacatggggaggcctgaccctcgtccttgtccagagctcctgccagggcctcggcgtcagactgagcctgcggcgggggagagaaggagaggagcgctgatccgggcacccagagttggggctgccttggagacaaatctggggcccccgagcaccaattgacaacgaaatctccccaggacaatgcgccgtagactgaaggacagggatggaagggcctattggagaggaagggacggccccaacttttaacacgcgcattctgggtgctgggagcggttaaagccaacattccctgccggaaaaccgaggctcagagaggggcggcgcccgccgggagtcccccagagcgtgagcagcagttcgtggccggaaaacctggccaggtccccagggccgggccgctggaggactgggcaccgcaggcagggccaaacggactcaccatggcgggcggcgcggtcccttcaagacagcgggtggtcgctttgcagccggaccctggctgggccatcacctgggggagggggggagggaacgcaggcggcggcggctgctg

SEQ ID NO: 19 - DNA, 1000 bp, Artificial Sequence
  Bisulfite modified sequence
cggtttagcgcgggttttttttatttcgggttttagttttttcggttttatttatagttagaggcgttgaagtttagaaggtgtatgcgatttttttatttttttttcgtaatattgagatttagggaaatggaaataaattttttttattttttagacggaattcgggggtttaggtagattttaagttttgtttaaagtttcgtagtcgggtagtagtggagttaggatttggaagtaagaggatttgcggtgtttttttgtagttttttgcgttgcgttttacgtttcgataatacgtacgtaatatttatttttgttttattttgagtagatatcggtttaggatttcgaggtcgtagttggagtagatgtttttgtttgtagacggtacggaggaggcggtagagggcggtgagtagatagatggcgtgttgggcgtatatggggaggtttgattttcgtttttgtttagagtttttgttagggtttcggcgttagattgagtttgcggcgggggagagaaggagaggagcgttgattcgggtatttagagttggggttgttttggagataaatttggggttttcgagtattaattgataacgaaatttttttaggataatgcgtcgtagattgaaggatagggatggaagggtttattggagaggaagggacggttttaatttttaatacgcgtattttgggtgttgggagcggttaaagttaatattttttgtcggaaaatcgaggtttagagaggggcggcgttcgtcgggagttttttagagcgtgagtagtagttcgtggtcggaaaatttggttaggtttttagggtcgggtcgttggaggattgggtatcgtaggtagggttaaacggatttattatggcgggcggcgcggtttttttaagatagcgggtggtcgttttgtagtcggattttggttgggttattatttgggggagggggggagggaacgtaggcggcggcggttgttg

SEQ ID NO: 20 - DNA, 20 bp, Artificial Sequence
  Primer
ggaattcgggggtttaggta

SEQ ID NO: 21 - DNA, 20 bp, Artificial Sequence
  Primer
acgctcctctccttctctcc

SEQ ID NO: 22 - DNA, 20 bp, Artificial Sequence
  Primer
gcgtatatggggaggtttga

SEQ ID NO: 23 - DNA, 23 bp, Artificial Sequence
  Primer
cctacgatacccaatcctccaac

SEQ ID NO: 24 - DNA, 4934 bp, Homo sapiens
ttgggagctcttggcctctctttgggcagagtgctccagtccacatcctaccagacccttgaccccgggcttcaggaaacagaagcctagagaacctcagcatgtgacccctccctgggccccagctccttagaggaaaattctgcctcccacgccaccattcacactctctccaggaagaacttcctcatagcagccacccagagcttgggctgcagtgcagtgcagacaatagtccttgcctggcactcgatcggctttttctttccctttttgtgggttttattatttttgttacaggtggggctgccagggatgggttatgcctgcagggggagaaatgatcagaagagccacaattctaccctcaacccagggaatgtgagcttttactgcctccattttcttaaccagaaatctggtttagttttgctttcagggctcttgtcattggaaaaagattagtgctcagaacctgcagcccagaaatggcccagtcccatccctccaggcaggctctgctcctcaagctgcgtggggaaatgccatcatgggcttgtgcccagcatccaccctgccaatgatgacaacagtgataatcgaggcattcataccaaccaccatttagggagcctttatagagacttccccccaacagtggcctctttggcagctctgggagacagccttggaaagggcgaactaagggccgagagaagcagcaacttgcgaaggtcactactggccagactgggcccagtctcctgcctcttcccacagtggctgcacaccctactctctaccccattgcagtaggaagagaactccagaataaggggaggctctgaacagtggagtcaggatccgtgttttgactagtttcaaggtctagtaaagcacagtatccaaggaggctcagtccagcatgggcatgggctagggctggagaagtagaaaagaaatttgggcaagtagtgaataagactgccaaatctattgttaggagagccaggagaggtgtcctagtggtgccttagtctatgggagagacccagacaccattctgctgggttcccaagctggcaccttaaatttagtagctgatgaatccaaggagcccccaagcatcatctggcatgtttttttgtatgtttgtttgtttgttttttgagacagagtctctctctgttacccaggctggagtgtagtgacgtgatcttggctcaccacaatgtccgcctcccaggttcaagtgattctcttgcctcagcctcctgagtagctgggactacaggcacgtgccaccacacctggctaagttttgtatttttagtagagatgggtttcaccatgttggccaggatggtctcgatctcctgaccttgtgatctaccagccttggcctcccaaagtgctgcgattataggtgtgagccaccacacccggcccatctggcatgttttataccaactggagtcaggcctagagcagggaggtggctagacagtgactgtaacctccatttcctgtcctggccaaaccaatactcagatgggacagtgagaggagacatcacactctggttacacaccattaacccctgtctgactacacacacacacacacacagccgtccagattcacaaatacgttcttatcacccccttcatccctcagtgcctgggtggaggcccttaagcaggaatgccccctcagaggagagggtgggagtggaatgatgggatttcagaatcccctcacctcaccctctcacctccagatcctagtccagatgtaatcctgtcctcaccactttgcgtgcacgtgcacgcacacacacatgcacacacacagtctcaacattcacatacagacacccactcttgacacccacacatgaactaaaagacaaacgttggtccataaaggaacacacatgctatctacatacccccaaccctgcccagtgatgctttccccagcactactgcacagatcccagacaatacagacacacaggcactccttgcacactgagtcctaggccacttggttgagctgcccccaccccaccccagctgcacactcttctacatccatcccataaaggaagagtccgtctctttaaccatgcttctcatggttttcagagtacccttgccccaaatgctgccaacctccccctagactcaagatcttctctttccagatcgctggaggctcaatgccagtgcacaggaggagatcgccttccaccatattccctgactcccagaggctctttctagggcaggggtctggccaggaagactgaagccatgacgtcttcctgtgcaaggataggaaagatgtctgtgggttggagggtagttatagggaagcagctttctccactttttgagaaagcacttgggaacaagcatccctctcaggaagtgattctccaccattctcctctgatcctataggcctggtggtccaagcctcaggccagttgatgcctcccactgggatcagcagacaaggccatgaccctgcagtgacctcgaccccataatcaggtcaggtccgggcttcatggctagaagcgaggcccaggcgagtggccaagacgcggcaggacaggaggatgcgcctggctgctctcggctgctggacgcggcctgcagtagggagagcgcagcccggggtaatcccactcagggctccgggtgcccagttctcccacttcccatcctggcggcctaaaggcaaggcctagaccctggagaggccaaagtcgggccaaaacaacagcgaagctgggactggaacaggcgctgggggcctgcgcatgaccccaggctcagaatgcgacactccagtgacgccggggaatgagttgagatggagccggagacagaggttggggttcaggacgaggcgcttgggtatgggatcggatctgagacggttgcggcgctggtgctttgggctggaccagactcgaacccagagcggagcgagggtcagagccagggcaagagtccgaagcccagctcagcgtccagcccgcgagagaccccaccatgaatgacgtccgagtagggttggaactcgaagcccgaacgcactggaaatgcagccggacgacggctgggatccgagtgggtccgggccagaaatggggacctcagagctccaccgaggcgctcgaggtcagaactgaagcctgagacttaggcaggacccgagacagagccagagacgataccgaaacccaatggaccgcgaggaccgaaggcagatccggggcgcaaacctgtgcaggcactggcgcgctgcctggagctctgggttcgcgccgctgagcgccggcaggttggaccagcgctgcgcgccggaagtgcactcgggacgccggggttctggaggagagaccacacgccgcaaaagtggcctccgaatgcgcccggggcctgccctcggcgacactgctggctcggcggccgcagcctacctgaagtagtccatcttgcagaagatctccttgttcttgatgtagcagctgttctgctgcctcagcgacgtgcgacacacggagcactcgaggcaccgcacgtgccagatgaggttgttgacctggggacggggcggggacggaggtcggctcagcgcgggcctctttcactccgggccccagccttcccggtctcatttacagtcagaggcgctgaagctcagaaggtgcatgcgattcccctatttttctcccgtaatactgagactcagggaaatggaaataaactcttcttatttttcagacggaacccgggggctcaggcagaccctaagtcttgcccaaagcttcgcagtcgggcagcagtggagccaggatttggaagtaagaggacctgcggtgcttccctgcagtctcctgcgctgcgtcccacgccccgacaacacgcacgcaacacctacccctgtctcaccttgagcagatatcggtccaggatctcgaggccgcagctggagcagatgttcttgcctgcagacggcacggaggaggcggcagagggcggtgagcagacagatggcgtgctgggcgtacatggggaggcctgaccctcgtccttgtccagagctcctgccagggcctcggcgtcagactgagcctgcggcgggggagagaaggagaggagcgctgatccgggcacccagagttggggctgccttggagacaaatctggggcccccgagcaccaattgacaacgaaatctccccaggacaatgcgccgtagactgaaggacagggatggaagggcctattggagaggaagggacggccccaacttttaacacgcgcattctgggtgctgggagcggttaaagccaacattccctgccggaaaaccgaggctcagagaggggcggcgcccgccgggagtcccccagagcgtgagcagcagttcgtggccggaaaacctggccaggtccccagggccgggccgctggaggactgggcaccgcaggcagggccaaacggactcaccatggcgggcggcgcggtcccttcaagacagcgggtggtcgctttgcagccggaccctggctgggccatcacctgggggagggggggagggaacgcaggcggcggcggctgctgaactggctccgcacagcctgagcccagcgcctccccgcgcctgttatataaaccggcgccgaacaatgagtcctaactttgtagtgggcatttaaagcccttccccacaaaagcggtgtctctctaatgaagcaatttgaatttggattggattttttccctctctctccccctctccctgcacttaacccgtggctcttgaagtaatcgcttagttcccttgcaatccaagcctctgaggggggaagaaaaacacgcgcacacacacacaaactacctgcaattaga

SEQ ID NO: 25 - DNA, 4934 bp, Artificial Sequence
  Bisulfite modified sequence
ttgggagtttttggtttttttttgggtagagtgttttagtttatattttattagatttttgatttcgggttttaggaaatagaagtttagagaattttagtatgtgatttttttttgggttttagttttttagaggaaaattttgttttttacgttattatttatattttttttaggaagaatttttttatagtagttatttagagtttgggttgtagtgtagtgtagataatagtttttgtttggtattcgatcggttttttttttttttttttgtgggttttattatttttgttataggtggggttgttagggatgggttatgtttgtagggggagaaatgattagaagagttataattttatttttaatttagggaatgtgagtttttattgtttttatttttttaattagaaatttggtttagttttgtttttagggtttttgttattggaaaaagattagtgtttagaatttgtagtttagaaatggtttagttttatttttttaggtaggttttgttttttaagttgcgtggggaaatgttattatgggtttgtgtttagtatttattttgttaatgatgataatagtgataatcgaggtatttatattaattattatttagggagtttttatagagatttttttttaatagtggtttttttggtagttttgggagatagttttggaaagggcgaattaagggtcgagagaagtagtaatttgcgaaggttattattggttagattgggtttagttttttgtttttttttatagtggttgtatattttattttttattttattgtagtaggaagagaattttagaataaggggaggttttgaatagtggagttaggattcgtgttttgattagttttaaggtttagtaaagtatagtatttaaggaggtttagtttagtatgggtatgggttagggttggagaagtagaaaagaaatttgggtaagtagtgaataagattgttaaatttattgttaggagagttaggagaggtgttttagtggtgttttagtttatgggagagatttagatattattttgttgggtttttaagttggtattttaaatttagtagttgatgaatttaaggagtttttaagtattatttggtatgtttttttgtatgtttgtttgtttgttttttgagatagagtttttttttgttatttaggttggagtgtagtgacgtgattttggtttattataatgttcgttttttaggtttaagtgatttttttgttttagttttttgagtagttgggattataggtacgtgttattatatttggttaagttttgtatttttagtagagatgggttttattatgttggttaggatggtttcgattttttgattttgtgatttattagttttggttttttaaagtgttgcgattataggtgtgagttattatattcggtttatttggtatgttttatattaattggagttaggtttagagtagggaggtggttagatagtgattgtaatttttattttttgttttggttaaattaatatttagatgggatagtgagaggagatattatattttggttatatattattaatttttgtttgattatatatatatatatatatagtcgtttagatttataaatacgtttttattattttttttattttttagtgtttgggtggaggtttttaagtaggaatgtttttttagaggagagggtgggagtggaatgatgggattttagaatttttttattttatttttttatttttagattttagtttagatgtaattttgtttttattattttgcgtgtacgtgtacgtatatatatatgtatatatatagttttaatatttatatatagatatttatttttgatatttatatatgaattaaaagataaacgttggtttataaaggaatatatatgttatttatatatttttaattttgtttagtgatgttttttttagtattattgtatagattttagataatatagatatataggtattttttgtatattgagttttaggttatttggttgagttgtttttattttattttagttgtatatttttttatatttattttataaaggaagagttcgtttttttaattatgttttttatggtttttagagtatttttgttttaaatgttgttaatttttttttagatttaagattttttttttttagatcgttggaggtttaatgttagtgtataggaggagatcgttttttattatattttttgatttttagaggttttttttagggtaggggtttggttaggaagattgaagttatgacgtttttttgtgtaaggataggaaagatgtttgtgggttggagggtagttatagggaagtagttttttttattttttgagaaagtatttgggaataagtattttttttaggaagtgattttttattatttttttttgattttataggtttggtggtttaagttttaggttagttgatgttttttattgggattagtagataaggttatgattttgtagtgatttcgattttataattaggttaggttcgggttttatggttagaagcgaggtttaggcgagtggttaagacgcggtaggataggaggatgcgtttggttgttttcggttgttggacgcggtttgtagtagggagagcgtagttcggggtaattttatttagggtttcgggtgtttagtttttttattttttattttggcggtttaaaggtaaggtttagattttggagaggttaaagtcgggttaaaataatagcgaagttgggattggaataggcgttgggggtttgcgtatgattttaggtttagaatgcgatattttagtgacgtcggggaatgagttgagatggagtcggagatagaggttggggtttaggacgaggcgtttgggtatgggatcggatttgagacggttgcggcgttggtgttttgggttggattagattcgaatttagagcggagcgagggttagagttagggtaagagttcgaagtttagtttagcgtttagttcgcgagagattttattatgaatgacgttcgagtagggttggaattcgaagttcgaacgtattggaaatgtagtcggacgacggttgggattcgagtgggttcgggttagaaatggggattttagagttttatcgaggcgttcgaggttagaattgaagtttgagatttaggtaggattcgagatagagttagagacgatatcgaaatttaatggatcgcgaggatcgaaggtagattcggggcgtaaatttgtgtaggtattggcgcgttgtttggagttttgggttcgcgtcgttgagcgtcggtaggttggattagcgttgcgcgtcggaagtgtattcgggacgtcggggttttggaggagagattatacgtcgtaaaagtggttttcgaatgcgttcggggtttgttttcggcgatattgttggttcggcggtcgtagtttatttgaagtagtttattttgtagaagatttttttgtttttgatgtagtagttgttttgttgttttagcgacgtgcgatatacggagtattcgaggtatcgtacgtgttagatgaggttgttgatttggggacggggcggggacggaggtcggtttagcgcgggttttttttatttcgggttttagttttttcggttttatttatagttagaggcgttgaagtttagaaggtgtatgcgatttttttatttttttttcgtaatattgagatttagggaaatggaaataaattttttttattttttagacggaattcgggggtttaggtagattttaagttttgtttaaagtttcgtagtcgggtagtagtggagttaggatttggaagtaagaggatttgcggtgtttttttgtagttttttgcgttgcgttttacgtttcgataatacgtacgtaatatttatttttgttttattttgagtagatatcggtttaggatttcgaggtcgtagttggagtagatgtttttgtttgtagacggtacggaggaggcggtagagggcggtgagtagatagatggcgtgttgggcgtatatggggaggtttgattttcgtttttgtttagagtttttgttagggtttcggcgttagattgagtttgcggcgggggagagaaggagaggagcgttgattcgggtatttagagttggggttgttttggagataaatttggggttttcgagtattaattgataacgaaatttttttaggataatgcgtcgtagattgaaggatagggatggaagggtttattggagaggaagggacggttttaatttttaatacgcgtattttgggtgttgggagcggttaaagttaatattttttgtcggaaaatcgaggtttagagaggggcggcgttcgtcgggagttttttagagcgtgagtagtagttcgtggtcggaaaatttggttaggtttttagggtcgggtcgttggaggattgggtatcgtaggtagggttaaacggatttattatggcgggcggcgcggtttttttaagatagcgggtggtcgttttgtagtcggattttggttgggttattatttgggggagggggggagggaacgtaggcggcggcggttgttgaattggtttcgtatagtttgagtttagcgttttttcgcgtttgttatataaatcggcgtcgaataatgagttttaattttgtagtgggtatttaaagtttttttttataaaagcggtgtttttttaatgaagtaatttgaatttggattggattttttttttttttttttttttttttttgtatttaattcgtggtttttgaagtaatcgtttagtttttttgtaatttaagtttttgaggggggaagaaaaatacgcgtatatatatataaattatttgtaattaga

SEQ ID NO: 26 - DNA, 22 bp, Artificial Sequence
  Primer
ttgggttgtagtgtagtgtaga

SEQ ID NO: 27 - DNA, 20 bp, Artificial Sequence
  Primer
aattcgccctttccaaaact

SEQ ID NO: 28 - DNA, 20 bp, Artificial Sequence
  Primer
gagagcgtagttcggggtaa

SEQ ID NO: 29 - DNA, 21 bp, Artificial Sequence
  Primer
tctcgcgaactaaacgctaaa

SEQ ID NO: 30 - DNA, 20 bp, Artificial Sequence
  Primer
aatttaatggatcgcgagga

SEQ ID NO: 31 - DNA, 20 bp, Artificial Sequence
  Primer
ccccaaatcaacaacctcat

SEQ ID NO: 32 - DNA, 20 bp, Artificial Sequence
  Primer
ggtgttgggagcggttaaag

SEQ ID NO: 33 - DNA, 20 bp, Artificial Sequence
  AAAACTCATTATTCGACGCC
aaaactcattattcgacgcc

SEQ ID NO: 34 - DNA, 804 bp, Homo sapiens
gagagatgggtacttcacgccacaaccccctcaaccaagaccacctccgcaaccacagcgggaaaagctaggggcaggcagcccacttttgcaattactctacattacagtgaactgcggtcctcacgtcttcttttcttcactccccttaacaaaataaaataaataatttcccttcctgcccacccacggttgcccaagaccaagtcttagaggcagccgggttccgatcaagtgctgcgaaacgacgcgtttgacagctgctctggagccgaggatcacaataagagaaggcgcgtgaggctccggcagcaaacaccagccaggcaggcagcggtaatcacagtgagcaaagttgaagactataaaagagccaggctaacgtgctgccgagcaggtgtcctggattttattgtagttgcaaatatgcttctggtgataagtatcgaaattattttttaagtgcgctggggaggagggaggtgcgggaattgagcctcctccgtttccagggagcctctgaaagtggggtggggggagatgaggcatgcacgcgaggcaaagacaaacaggaaagtgtctctatcgggaccaacgtgtgcgaccctacctgaaacggcaagcagaattcggtgttttcttccttttgccctgatcttgacgagataggaaacttgggagagagagagagagagagagagagagagagagagagagagagagagagagagagagagaccgagactgcagcagccaagagagcgtggagcgatgggctggtggaagccggagaggagcgctagg

SEQ ID NO: 35 - DNA, 804 bp, Artificial Sequence
  Bisulfite modified sequence
gagagatgggtattttacgttataatttttttaattaagattattttcgtaattatagcgggaaaagttaggggtaggtagtttatttttgtaattattttatattatagtgaattgcggtttttacgtttttttttttttattttttttaataaaataaaataaataatttttttttttgtttatttacggttgtttaagattaagttttagaggtagtcgggtttcgattaagtgttgcgaaacgacgcgtttgatagttgttttggagtcgaggattataataagagaaggcgcgtgaggtttcggtagtaaatattagttaggtaggtagcggtaattatagtgagtaaagttgaagattataaaagagttaggttaacgtgttgtcgagtaggtgttttggattttattgtagttgtaaatatgtttttggtgataagtatcgaaattattttttaagtgcgttggggaggagggaggtgcgggaattgagtttttttcgtttttagggagtttttgaaagtggggtggggggagatgaggtatgtacgcgaggtaaagataaataggaaagtgtttttatcgggattaacgtgtgcgattttatttgaaacggtaagtagaattcggtgtttttttttttttgttttgattttgacgagataggaaatttgggagagagagagagagagagagagagagagagagagagagagagagagagagagagagagatcgagattgtagtagttaagagagcgtggagcgatgggttggtggaagtcggagaggagcgttagg

SEQ ID NO: 36 - DNA, 21 bp, Artificial Sequence
  Primer
tcgggtttcgattaagtgttg

SEQ ID NO: 37 - DNA, 20 bp, Artificial Sequence
  Primer
tttcaaataaaatcgcacac